European Patent Specification EP 3 638 243 B1, published August 7, 2024. Title: METHODS FOR TREATING MYELOPROLIFERATIVE NEOPLASM-ASSOCIATED MYELOFIBROSIS AND ANEMIA. Applicant: CELGENE CORPORATION. Application To Be Assigned. The sequence listing filed with the application follows.

SEQUENCE LISTING (34 sequences)

SEQ ID NO: 1 - protein, 344 aa, Homo sapiens
  Extracellular domain of human ActRIIA fused to a human Fc domain
ILGRSETQECLFFNANWEKDRTNQTGVEPCYGDKDKRRHCFATWKNISGSIEIVKQGCWLDDINCYDRTDCVEKKDSPEVYFCCCEGNMCNEKFSYFPEMEVTQPTSNPVTPKPPTGGGTHTCPPCPAPELLGGPSVFLFPPKPKDTLMISRTPEVTCVVVDVSHEDPEVKFNWYVDGVEVHNAKTKPREEQYNSTYRVVSVLTVLHQDWLNGKEYKCKVSNKALPVPIEKTISKAKGQPREPQVYTLPPSREEMTKNQVSLTCLVKGFYPSDIAVEWESNGQPENNYKTTPPVLDSDGSFFLYSKLTVDKSRWQQGNVFSCSVMHEALHNHYTQKSLSLSPGK

SEQ ID NO: 2 - protein, 21 aa, Artificial Sequence
  Leader sequence of Honey bee mellitin (HBML)
MKFLVNVALVFMVVYISYIYA

SEQ ID NO: 3 - protein, 512 aa, Homo sapiens
  human ActRIIB precursor protein sequence (A64)
MTAPWVALALLWGSLWPGSGRGEAETRECIYYNANWELERTNQSGLERCEGEQDKRLHCYASWANSSGTIELVKKGCWLDDFNCYDRQECVATEENPQVYFCCCEGNFCNERFTHLPEAGGPEVTYEPPPTAPTLLTVLAYSLLPIGGLSLIVLLAFWMYRHRKPPYGHVDIHEDPGPPPPSPLVGLKPLQLLEIKARGRFGCVWKAQLMNDFVAVKIFPLQDKQSWQSEREIFSTPGMKHENLLQFIAAEKRGSNLEVELWLITAFHDKGSLTDYLKGNIITWNELCHVAETMSRGLSYLHEDVPWCRGEGHKPSIAHRDFKSKNVLLKSDLTAVLADFGLAVRFEPGKPPGDTHGQVGTRRYMAPEVLEGAINFQRDAFLRIDMYAMGLVLWELVSRCKAADGPVDEYMLPFEEEIGQHPSLEELQEVVVHKKMRPTIKDHWLKHPGLAQLCVTIEECWDHDAEARLSAGCVEERVSLIRRSVNGTTSDCLVSLVTSVTNVDLPPKESSI

SEQ ID NO: 4 - protein, 116 aa, Homo sapiens
  human ActRIIB soluble (extracellular), processed polypeptide sequence (amino acids 19-134 of SEQ ID NO:3)
SGRGEAETRECIYYNANWELERTNQSGLERCEGEQDKRLHCYASWANSSGTIELVKKGCWLDDFNCYDRQECVATEENPQVYFCCCEGNFCNERFTHLPEAGGPEVTYEPPPTAPT

SEQ ID NO: 5 - protein, 101 aa, Homo sapiens
  human ActRIIB soluble (extracellular), processed polypeptide sequence with the C-terminal 15 amino acids deleted (amino acids 19-119 of SEQ ID NO:3)
SGRGEAETRECIYYNANWELERTNQSGLERCEGEQDKRLHCYASWANSSGTIELVKKGCWLDDFNCYDRQECVATEENPQVYFCCCEGNFCNERFTHLPEA

SEQ ID NO: 6 - DNA, 1539 bp, Homo sapiens
  human ActRIIB (A64) precursor protein
atgacggcgccctgggtggccctcgccctcctctggggatcgctgtggcccggctctgggcgtggggaggctgagacacgggagtgcatctactacaacgccaactgggagctggagcgcaccaaccagagcggcctggagcgctgcgaaggcgagcaggacaagcggctgcactgctacgcctcctgggccaacagctctggcaccatcgagctcgtgaagaagggctgctggctagatgacttcaactgctacgataggcaggagtgtgtggccactgaggagaacccccaggtgtacttctgctgctgtgaaggcaacttctgcaacgagcgcttcactcatttgccagaggctgggggcccggaagtcacgtacgagccacccccgacagcccccaccctgctcacggtgctggcctactcactgctgcccatcgggggcctttccctcatcgtcctgctggccttttggatgtaccggcatcgcaagcccccctacggtcatgtggacatccatgaggaccctgggcctccaccaccatcccctctggtgggcctgaagccactgcagctgctggagatcaaggctcgggggcgctttggctgtgtctggaaggcccagctcatgaatgactttgtagctgtcaagatcttcccactccaggacaagcagtcgtggcagagtgaacgggagatcttcagcacacctggcatgaagcacgagaacctgctacagttcattgctgccgagaagcgaggctccaacctcgaagtagagctgtggctcatcacggccttccatgacaagggctccctcacggattacctcaaggggaacatcatcacatggaacgaactgtgtcatgtagcagagacgatgtcacgaggcctctcatacctgcatgaggatgtgccctggtgccgtggcgagggccacaagccgtctattgcccacagggactttaaaagtaagaatgtattgctgaagagcgacctcacagccgtgctggctgactttggcttggctgttcgatttgagccagggaaacctccaggggacacccacggacaggtaggcacgagacggtacatggctcctgaggtgctcgagggagccatcaacttccagagagatgccttcctgcgcattgacatgtatgccatggggttggtgctgtgggagcttgtgtctcgctgcaaggctgcagacggacccgtggatgagtacatgctgccctttgaggaagagattggccagcacccttcgttggaggagctgcaggaggtggtggtgcacaagaagatgaggcccaccattaaagatcactggttgaaacacccgggcctggcccagctttgtgtgaccatcgaggagtgctgggaccatgatgcagaggctcgcttgtccgcgggctgtgtggaggagcgggtgtccctgattcggaggtcggtcaacggcactacctcggactgtctcgtttccctggtgacctctgtcaccaatgtggacctgccccctaaagagtcaagcatctaa

SEQ ID NO: 7 - protein, 344 aa, Artificial Sequence
  fusion protein comprising a soluble extracellular domain of ActRIIB (A64; SEQ ID NO:17) fused to an Fc domain
SGRGEAETRECIYYNANWELERTNQSGLERCEGEQDKRLHCYASWANSSGTIELVKKGCWLDDFNCYDRQECVATEENPQVYFCCCEGNFCNERFTHLPEAGGPEVTYEPPPTAPTGGGTHTCPPCPAPELLGGPSVFLFPPKPKDTLMISRTPEVTCVVVDVSHEDPEVKFNWYVDGVEVHNAKTKPREEQYNSTYRVVSVLTVLHQDWLNGKEYKCKVSNKALPVPIEKTISKAKGQPREPQVYTLPPSREEMTKNQVSLTCLVKGFYPSDIAVEWESNGQPENNYKTTPPVLDSDGSFFLYSKLTVDKSRWQQGNVFSCSVMHEALHNHYTQKSLSLSPGK

SEQ ID NO: 8 - protein, 329 aa, Artificial Sequence
  fusion protein comprising a soluble extracellular domain of ActRIIB (A64) with the C-terminal 15 amino acids deleted (SEQ ID NO:5) fused to an Fc domain
SGRGEAETRECIYYNANWELERTNQSGLERCEGEQDKRLHCYASWANSSGTIELVKKGCWLDDFNCYDRQECVATEENPQVYFCCCEGNFCNERFTHLPEAGGGTHTCPPCPAPELLGGPSVFLFPPKPKDTLMISRTPEVTCVVVDVSHEDPEVKFNWYVDGVEVHNAKTKPREEQYNSTYRVVSVLTVLHQDWLNGKEYKCKVSNKALPVPIEKTISKAKGQPREPQVYTLPPSREEMTKNQVSLTCLVKGFYPSDIAVEWESNGQPENNYKTTPPVLDSDGSFFLYSKLTVDKSRWQQGNVFSCSVMHEALHNHYTQKSLSLSPGK

SEQ ID NO: 9 - protein, 107 aa, Homo sapiens
  human ActRIIB soluble (extracellular), processed polypeptide sequence with the N-terminal 6 amino acids of the EC domain deleted and the C-terminal 3 amino acids of the EC domain deleted (amino acids 25-131 of SEQ ID NO:14) and with an L79D mutation
ETRECIYYNANWELERTNQSGLERCEGEQDKRLHCYASWRNSSGTIELVKKGCWDDDFNCYDRQECVATEENPQVYFCCCEGNFCNERFTHLPEAGGPEVTYEPPPT

SEQ ID NO: 10 - protein, 360 aa, Artificial Sequence
  Unprocessed ActRIIB-Fc fusion protein with the N-terminal 6 amino acids of the EC domain deleted and the C-terminal 3 amino acids of the EC domain deleted (amino acids 25-131 of SEQ ID NO:14) and with an L79D mutation and with TPA leader sequence
MDAMKRGLCCVLLLCGAVFVSPGAAETRECIYYNANWELERTNQSGLERCEGEQDKRLHCYASWRNSSGTIELVKKGCWDDDFNCYDRQECVATEENPQVYFCCCEGNFCNERFTHLPEAGGPEVTYEPPPTGGGTHTCPPCPAPELLGGPSVFLFPPKPKDTLMISRTPEVTCVVVDVSHEDPEVKFNWYVDGVEVHNAKTKPREEQYNSTYRVVSVLTVLHQDWLNGKEYKCKVSNKALPAPIEKTISKAKGQPREPQVYTLPPSREEMTKNQVSLTCLVKGFYPSDIAVEWESNGQPENNYKTTPPVLDSDGSFFLYSKLTVDKSRWQQGNVFSCSVMHEALHNHYTQKSLSLSPGK

SEQ ID NO: 11 - protein, 335 aa, Artificial Sequence
  Processed ActRIIB-Fc fusion protein with the N-terminal 6 amino acids of the EC domain deleted and the C-terminal 3 amino acids of the EC domain deleted (amino acids 25-131 of SEQ ID NO:14) and with an L79D mutation (i.e., luspatercept)
ETRECIYYNANWELERTNQSGLERCEGEQDKRLHCYASWRNSSGTIELVKKGCWDDDFNCYDRQECVATEENPQVYFCCCEGNFCNERFTHLPEAGGPEVTYEPPPTGGGTHTCPPCPAPELLGGPSVFLFPPKPKDTLMISRTPEVTCVVVDVSHEDPEVKFNWYVDGVEVHNAKTKPREEQYNSTYRVVSVLTVLHQDWLNGKEYKCKVSNKALPAPIEKTISKAKGQPREPQVYTLPPSREEMTKNQVSLTCLVKGFYPSDIAVEWESNGQPENNYKTTPPVLDSDGSFFLYSKLTVDKSRWQQGNVFSCSVMHEALHNHYTQKSLSLSPGK

SEQ ID NO: 12 - protein, 115 aa, Homo sapiens
  human ActRIIB soluble (extracellular), processed polypeptide sequence (amino acids 20-134 of SEQ ID NO:3)
GRGEAETRECIYYNANWELERTNQSGLERCEGEQDKRLHCYASWANSSGTIELVKKGCWLDDFNCYDRQECVATEENPQVYFCCCEGNFCNERFTHLPEAGGPEVTYEPPPTAPT

SEQ ID NO: 13 - protein, 100 aa, Homo sapiens
  human ActRIIB soluble (extracellular), processed polypeptide sequence with the C-terminal 15 amino acids deleted (amino acids 20-119 of SEQ ID NO:3)
GRGEAETRECIYYNANWELERTNQSGLERCEGEQDKRLHCYASWANSSGTIELVKKGCWLDDFNCYDRQECVATEENPQVYFCCCEGNFCNERFTHLPEA

SEQ ID NO: 14 - protein, 512 aa, Homo sapiens
  human ActRIIB precursor protein sequence (R64)
MTAPWVALALLWGSLWPGSGRGEAETRECIYYNANWELERTNQSGLERCEGEQDKRLHCYASWRNSSGTIELVKKGCWLDDFNCYDRQECVATEENPQVYFCCCEGNFCNERFTHLPEAGGPEVTYEPPPTAPTLLTVLAYSLLPIGGLSLIVLLAFWMYRHRKPPYGHVDIHEDPGPPPPSPLVGLKPLQLLEIKARGRFGCVWKAQLMNDFVAVKIFPLQDKQSWQSEREIFSTPGMKHENLLQFIAAEKRGSNLEVELWLITAFHDKGSLTDYLKGNIITWNELCHVAETMSRGLSYLHEDVPWCRGEGHKPSIAHRDFKSKNVLLKSDLTAVLADFGLAVRFEPGKPPGDTHGQVGTRRYMAPEVLEGAINFQRDAFLRIDMYAMGLVLWELVSRCKAADGPVDEYMLPFEEEIGQHPSLEELQEVVVHKKMRPTIKDHWLKHPGLAQLCVTIEECWDHDAEARLSAGCVEERVSLIRRSVNGTTSDCLVSLVTSVTNVDLPPKESSI

SEQ ID NO: 15 - protein, 116 aa, Homo sapiens
  human ActRIIB soluble (extracellular), processed polypeptide sequence (amino acids 19-134 of SEQ ID NO:14)
SGRGEAETRECIYYNANWELERTNQSGLERCEGEQDKRLHCYASWRNSSGTIELVKKGCWLDDFNCYDRQECVATEENPQVYFCCCEGNFCNERFTHLPEAGGPEVTYEPPPTAPT

SEQ ID NO: 16 - protein, 101 aa, Homo sapiens
  human ActRIIB soluble (extracellular), processed polypeptide sequence with the C-terminal 15 amino acids deleted (amino acids 19-119 of SEQ ID NO:14)
SGRGEAETRECIYYNANWELERTNQSGLERCEGEQDKRLHCYASWRNSSGTIELVKKGCWLDDFNCYDRQECVATEENPQVYFCCCEGNFCNERFTHLPEA

SEQ ID NO: 17 - protein, 115 aa, Homo sapiens
  human ActRIIB soluble (extracellular), processed polypeptide sequence (amino acids 20-134 of SEQ ID NO:14)
GRGEAETRECIYYNANWELERTNQSGLERCEGEQDKRLHCYASWRNSSGTIELVKKGCWLDDFNCYDRQECVATEENPQVYFCCCEGNFCNERFTHLPEAGGPEVTYEPPPTAPT

SEQ ID NO: 18 - protein, 100 aa, Homo sapiens
  human ActRIIB soluble (extracellular), processed polypeptide sequence with the C-terminal 15 amino acids deleted (amino acids 20-119 of SEQ ID NO:14)
GRGEAETRECIYYNANWELERTNQSGLERCEGEQDKRLHCYASWRNSSGTIELVKKGCWLDDFNCYDRQECVATEENPQVYFCCCEGNFCNERFTHLPEA

SEQ ID NO: 19 - protein, 107 aa, Homo sapiens
  human ActRIIB soluble (extracellular), processed polypeptide sequence with the N-terminal 6 amino acids of the EC domain deleted and the C-terminal 3 amino acids of the EC domain deleted (amino acids 25-131 of SEQ ID NO:3) and with an L79D mutation
ETRECIYYNANWELERTNQSGLERCEGEQDKRLHCYASWANSSGTIELVKKGCWDDDFNCYDRQECVATEENPQVYFCCCEGNFCNERFTHLPEAGGPEVTYEPPPT

SEQ ID NO: 20 - protein, 360 aa, Artificial Sequence
  Unprocessed ActRIIB-Fc fusion protein with the N-terminal 6 amino acids of the EC domain deleted and the C-terminal 3 amino acids of the EC domain deleted (amino acids 25-131 of SEQ ID NO:3) and with an L79D mutation and with TPA leader sequence
MDAMKRGLCCVLLLCGAVFVSPGAAETRECIYYNANWELERTNQSGLERCEGEQDKRLHCYASWANSSGTIELVKKGCWDDDFNCYDRQECVATEENPQVYFCCCEGNFCNERFTHLPEAGGPEVTYEPPPTGGGTHTCPPCPAPELLGGPSVFLFPPKPKDTLMISRTPEVTCVVVDVSHEDPEVKFNWYVDGVEVHNAKTKPREEQYNSTYRVVSVLTVLHQDWLNGKEYKCKVSNKALPAPIEKTISKAKGQPREPQVYTLPPSREEMTKNQVSLTCLVKGFYPSDIAVEWESNGQPENNYKTTPPVLDSDGSFFLYSKLTVDKSRWQQGNVFSCSVMHEALHNHYTQKSLSLSPGK

SEQ ID NO: 21 - protein, 335 aa, Artificial Sequence
  Processed ActRIIB-Fc fusion protein with the N-terminal 6 amino acids of the EC domain deleted and the C-terminal 3 amino acids of the EC domain deleted (amino acids 25-131 of SEQ ID NO:3) and with an L79D mutation
ETRECIYYNANWELERTNQSGLERCEGEQDKRLHCYASWANSSGTIELVKKGCWDDDFNCYDRQECVATEENPQVYFCCCEGNFCNERFTHLPEAGGPEVTYEPPPTGGGTHTCPPCPAPELLGGPSVFLFPPKPKDTLMISRTPEVTCVVVDVSHEDPEVKFNWYVDGVEVHNAKTKPREEQYNSTYRVVSVLTVLHQDWLNGKEYKCKVSNKALPAPIEKTISKAKGQPREPQVYTLPPSREEMTKNQVSLTCLVKGFYPSDIAVEWESNGQPENNYKTTPPVLDSDGSFFLYSKLTVDKSRWQQGNVFSCSVMHEALHNHYTQKSLSLSPGK

SEQ ID NO: 22 - protein, 115 aa, Homo sapiens
  human ActRIIB soluble (extracellular), processed polypeptide sequence (amino acids 20-134 of SEQ ID NO:14) with L79D mutation
GRGEAETRECIYYNANWELERTNQSGLERCEGEQDKRLHCYASWRNSSGTIELVKKGCWDDDFNCYDRQECVATEENPQVYFCCCEGNFCNERFTHLPEAGGPEVTYEPPPTAPT

SEQ ID NO: 23 - protein, 115 aa, Homo sapiens
  human ActRIIB soluble (extracellular), processed polypeptide sequence (amino acids 20-134 of SEQ ID NO:3) with L79D mutation
GRGEAETRECIYYNANWELERTNQSGLERCEGEQDKRLHCYASWANSSGTIELVKKGCWDDDFNCYDRQECVATEENPQVYFCCCEGNFCNERFTHLPEAGGPEVTYEPPPTAPT

SEQ ID NO: 24 - protein, 343 aa, Homo sapiens
  human ActRIIB soluble (extracellular), processed polypeptide sequence (amino acids 20-134 of SEQ ID NO:14) with L79D mutation fused to an Fc domain with a GGG linker
GRGEAETRECIYYNANWELERTNQSGLERCEGEQDKRLHCYASWRNSSGTIELVKKGCWDDDFNCYDRQECVATEENPQVYFCCCEGNFCNERFTHLPEAGGPEVTYEPPPTAPTGGGTHTCPPCPAPELLGGPSVFLFPPKPKDTLMISRTPEVTCVVVDVSHEDPEVKFNWYVDGVEVHNAKTKPREEQYNSTYRVVSVLTVLHQDWLNGKEYKCKVSNKALPAPIEKTISKAKGQPREPQVYTLPPSREEMTKNQVSLTCLVKGFYPSDIAVEWESNGQPENNYKTTPPVLDSDGSFFLYSKLTVDKSRWQQGNVFSCSVMHEALHNHYTQKSLSLSPGK

SEQ ID NO: 25 - protein, 343 aa, Homo sapiens
  human ActRIIB soluble (extracellular), processed polypeptide sequence (amino acids 20-134 of SEQ ID NO:3) with L79D mutation fused to an Fc domain
GRGEAETRECIYYNANWELERTNQSGLERCEGEQDKRLHCYASWANSSGTIELVKKGCWDDDFNCYDRQECVATEENPQVYFCCCEGNFCNERFTHLPEAGGPEVTYEPPPTAPTGGGTHTCPPCPAPELLGGPSVFLFPPKPKDTLMISRTPEVTCVVVDVSHEDPEVKFNWYVDGVEVHNAKTKPREEQYNSTYRVVSVLTVLHQDWLNGKEYKCKVSNKALPAPIEKTISKAKGQPREPQVYTLPPSREEMTKNQVSLTCLVKGFYPSDIAVEWESNGQPENNYKTTPPVLDSDGSFFLYSKLTVDKSRWQQGNVFSCSVMHEALHNHYTQKSLSLSPGK

SEQ ID NO: 26 - protein, 368 aa, Homo sapiens
  human ActRIIB soluble (extracellular), processed polypeptide sequence (amino acids 20-134 of SEQ ID NO:14) with L79D mutation fused to an Fc domain and with TPA leader sequence
MDAMKRGLCCVLLLCGAVFVSPGASGRGEAETRECIYYNANWELERTNQSGLERCEGEQDKRLHCYASWRNSSGTIELVKKGCWDDDFNCYDRQECVATEENPQVYFCCCEGNFCNERFTHLPEAGGPEVTYEPPPTAPTGGGTHTCPPCPAPELLGGPSVFLFPPKPKDTLMISRTPEVTCVVVDVSHEDPEVKFNWYVDGVEVHNAKTKPREEQYNSTYRVVSVLTVLHQDWLNGKEYKCKVSNKALPAPIEKTISKAKGQPREPQVYTLPPSREEMTKNQVSLTCLVKGFYPSDIAVEWESNGQPENNYKTTPPVLDSDGSFFLYSKLTVDKSRWQQGNVFSCSVMHEALHNHYTQKSLSLSPGK

SEQ ID NO: 27 - protein, 368 aa, Homo sapiens
  human ActRIIB soluble (extracellular), processed polypeptide sequence (amino acids 20-134 of SEQ ID NO:3) with L79D mutation fused to an Fc domain and with TPA leader sequence
MDAMKRGLCCVLLLCGAVFVSPGASGRGEAETRECIYYNANWELERTNQSGLERCEGEQDKRLHCYASWANSSGTIELVKKGCWDDDFNCYDRQECVATEENPQVYFCCCEGNFCNERFTHLPEAGGPEVTYEPPPTAPTGGGTHTCPPCPAPELLGGPSVFLFPPKPKDTLMISRTPEVTCVVVDVSHEDPEVKFNWYVDGVEVHNAKTKPREEQYNSTYRVVSVLTVLHQDWLNGKEYKCKVSNKALPAPIEKTISKAKGQPREPQVYTLPPSREEMTKNQVSLTCLVKGFYPSDIAVEWESNGQPENNYKTTPPVLDSDGSFFLYSKLTVDKSRWQQGNVFSCSVMHEALHNHYTQKSLSLSPGK

SEQ ID NO: 28 - protein, 141 aa, Homo sapiens
  human ActRIIB soluble (extracellular), processed polypeptide sequence having a variant C-terminal sequence (disclosed in WO2007/053775)
GRGEAETRECIYYNANWELERTNQSGLERCEGEQDKRLHCYASWRNSSGTIELVKKGCWLDDFNCYDRQECVATEENPQVYFCCCEGNFCNERFTHLPEAGGPEGPWASTTIPSGGPEATAAAGDQGSGALWLCLEGPAHE

SEQ ID NO: 29 - protein, 141 aa, Homo sapiens
  human ActRIIB soluble (extracellular), processed polypeptide sequence having a variant C-terminal sequence (disclosed in WO2007/053775) having an L79D mutation
GRGEAETRECIYYNANWELERTNQSGLERCEGEQDKRLHCYASWRNSSGTIELVKKGCWDDDFNCYDRQECVATEENPQVYFCCCEGNFCNERFTHLPEAGGPEGPWASTTIPSGGPEATAAAGDQGSGALWLCLEGPAHE

SEQ ID NO: 30 - protein, 370 aa, Homo sapiens
  human ActRIIB soluble (extracellular), processed polypeptide sequence having a variant C-terminal sequence (disclosed in WO2007/053775) having an L79D mutation fused to an Fc domain with a TGGG linker
GRGEAETRECIYYNANWELERTNQSGLERCEGEQDKRLHCYASWRNSSGTIELVKKGCWDDDFNCYDRQECVATEENPQVYFCCCEGNFCNERFTHLPEAGGPEGPWASTTIPSGGPEATAAAGDQGSGALWLCLEGPAHETGGGTHTCPPCPAPELLGGPSVFLFPPKPKDTLMISRTPEVTCVVVDVSHEDPEVKFNWYVDGVEVHNAKTKPREEQYNSTYRVVSVLTVLHQDWLNGKEYKCKVSNKALPAPIEKTISKAKGQPREPQVYTLPPSREEMTKNQVSLTCLVKGFYPSDIAVEWESNGQPENNYKTTPPVLDSDGSFFLYSKLTVDKSRWQQGNVFSCSVMHEALHNHYTQKSLSLSPGK

SEQ ID NO: 31 - DNA, 1083 bp, Artificial Sequence
  Nucleic Acid Sequence Encoding SEQ ID NO:10
atggatgcaatgaagagagggctctgctgtgtgctgctgctgtgtggagcagtcttcgtttcgcccggcgccgccgaaacccgcgaatgtatttattacaatgctaattgggaactcgaacggacgaaccaatccgggctcgaacggtgtgagggggaacaggataaacgcctccattgctatgcgtcgtggaggaactcctccgggacgattgaactggtcaagaaagggtgctgggacgacgatttcaattgttatgaccgccaggaatgtgtcgcgaccgaagagaatccgcaggtctatttctgttgttgcgaggggaatttctgtaatgaacggtttacccacctccccgaagccggcgggcccgaggtgacctatgaacccccgcccaccggtggtggaactcacacatgcccaccgtgcccagcacctgaactcctggggggaccgtcagtcttcctcttccccccaaaacccaaggacaccctcatgatctcccggacccctgaggtcacatgcgtggtggtggacgtgagccacgaagaccctgaggtcaagttcaactggtacgtggacggcgtggaggtgcataatgccaagacaaagccgcgggaggagcagtacaacagcacgtaccgtgtggtcagcgtcctcaccgtcctgcaccaggactggctgaatggcaaggagtacaagtgcaaggtctccaacaaagccctcccagcccccatcgagaaaaccatctccaaagccaaagggcagccccgagaaccacaggtgtacaccctgcccccatcccgggaggagatgaccaagaaccaggtcagcctgacctgcctggtcaaaggcttctatcccagcgacatcgccgtggagtgggagagcaatgggcagccggagaacaactacaagaccacgcctcccgtgctggactccgacggctccttcttcctctatagcaagctcaccgtggacaagagcaggtggcagcaggggaacgtcttctcatgctccgtgatgcatgaggctctgcacaaccactacacgcagaagagcctctccctgtccccgggtaaatga

SEQ ID NO: 32 - protein, 344 aa, Artificial Sequence
  fusion protein comprising a soluble extracellular domain of ActRIIB (R64; SEQ ID NO:15) fused to an Fc domain
SGRGEAETRECIYYNANWELERTNQSGLERCEGEQDKRLHCYASWRNSSGTIELVKKGCWLDDFNCYDRQECVATEENPQVYFCCCEGNFCNERFTHLPEAGGPEVTYEPPPTAPTGGGTHTCPPCPAPELLGGPSVFLFPPKPKDTLMISRTPEVTCVVVDVSHEDPEVKFNWYVDGVEVHNAKTKPREEQYNSTYRVVSVLTVLHQDWLNGKEYKCKVSNKALPVPIEKTISKAKGQPREPQVYTLPPSREEMTKNQVSLTCLVKGFYPSDIAVEWESNGQPENNYKTTPPVLDSDGSFFLYSKLTVDKSRWQQGNVFSCSVMHEALHNHYTQKSLSLSPGK

SEQ ID NO: 33 - protein, 329 aa, Artificial Sequence
  fusion protein comprising a soluble extracellular domain of ActRIIB (R64) with the C-terminal 15 amino acids deleted (SEQ ID NO:16) fused to an Fc domain
SGRGEAETRECIYYNANWELERTNQSGLERCEGEQDKRLHCYASWRNSSGTIELVKKGCWLDDFNCYDRQECVATEENPQVYFCCCEGNFCNERFTHLPEAGGGTHTCPPCPAPELLGGPSVFLFPPKPKDTLMISRTPEVTCVVVDVSHEDPEVKFNWYVDGVEVHNAKTKPREEQYNSTYRVVSVLTVLHQDWLNGKEYKCKVSNKALPVPIEKTISKAKGQPREPQVYTLPPSREEMTKNQVSLTCLVKGFYPSDIAVEWESNGQPENNYKTTPPVLDSDGSFFLYSKLTVDKSRWQQGNVFSCSVMHEALHNHYTQKSLSLSPGK

SEQ ID NO: 34 - protein, 344 aa, Homo sapiens; identical to SEQ ID NO: 1
  Extracellular domain of human ActRIIA fused to a human Fc domain